European Patent Specification EP 3 719 126 B1, published January 1, 2025. Title: NUCLEIC ACID, COMPOSITION AND CONJUGATE CONTAINING NUCLEIC ACID, PREPARATION METHOD THEREFOR AND USE THEREOF. Applicant: SUZHOU RIBO LIFE SCIENCE CO., LTD. Application 18 883 803.1. The sequence listing filed with the application follows.

SEQUENCE LISTING (64 sequences)

SEQ ID NO: 1 - RNA, 19 nt, Artificial Sequence
  misc_feature (19)..(19): n is Z, Z is A
ccaagagcaccaagaacun

SEQ ID NO: 2 - RNA, 19 nt, Artificial Sequence
  misc_feature (1)..(1): n is Z', Z'is U
naguucuuggugcucuugg

SEQ ID NO: 3 - RNA, 19 nt, Artificial Sequence
  misc_feature (19)..(19): n is ZA, ZA is A, U, G or C
ccaagagcaccaagaacun

SEQ ID NO: 4 - RNA, 19 nt, Artificial Sequence
  misc_feature (1)..(1): n is Z'B, Z'B is a neucleotide complementary to ZA, ZA is selected from A, U, G or C
naguucuuggugcucuugg

SEQ ID NO: 5 - RNA, 21 nt, Artificial Sequence
  misc_feature (1)..(1): n is Z'B, Z'B is a neucleotide complementary to ZA, ZA is selected from A, U, G or C
naguucuuggugcucuuggcu

SEQ ID NO: 6 - RNA, 21 nt, Artificial Sequence
  misc_feature (21)..(21): n is ZA, ZA is selected from A、U、G or C
agccaagagcaccaagaacun

SEQ ID NO: 7 - RNA, 23 nt, Artificial Sequence
  misc_feature (1)..(1): n is Z'B, Z'B is a neucleotide complementary to ZA, ZA is selected from A, U, G or C
naguucuuggugcucuuggcuug

SEQ ID NO: 8 - RNA, 19 nt, Artificial Sequence
ccaagagcaccaagaacua

SEQ ID NO: 9 - RNA, 21 nt, Artificial Sequence
uaguucuuggugcucuuggcu

SEQ ID NO: 10 - RNA, 21 nt, Artificial Sequence
agccaagagcaccaagaacua

SEQ ID NO: 11 - RNA, 23 nt, Artificial Sequence
uaguucuuggugcucuuggcuug

SEQ ID NO: 12 - RNA, 19 nt, Artificial Sequence
ccaagagcaccaagaacua

SEQ ID NO: 13 - RNA, 21 nt, Artificial Sequence
uaguucuuggugcucuuggcu

SEQ ID NO: 14 - RNA, 21 nt, Artificial Sequence
agccaagagcaccaagaacua

SEQ ID NO: 15 - RNA, 23 nt, Artificial Sequence
uaguucuuggugcucuuggcuug

SEQ ID NO: 16 - RNA, 21 nt, Artificial Sequence
uaguucuuggugcucuuggcu

SEQ ID NO: 17 - RNA, 23 nt, Artificial Sequence
uaguucuuggugcucuuggcuug

SEQ ID NO: 18 - RNA, 19 nt, Artificial Sequence
ccaagagcaccaagaacua

SEQ ID NO: 19 - RNA, 21 nt, Artificial Sequence
agccaagagcaccaagaacua

SEQ ID NO: 20 - RNA, 19 nt, Artificial Sequence
ccaagagcaccaagaacua

SEQ ID NO: 21 - RNA, 21 nt, Artificial Sequence
uaguucuuggugcucuuggcu

SEQ ID NO: 22 - RNA, 21 nt, Artificial Sequence
agccaagagcaccaagaacua

SEQ ID NO: 23 - RNA, 23 nt, Artificial Sequence
uaguucuuggugcucuuggcuug

SEQ ID NO: 24 - RNA, 21 nt, Artificial Sequence
uaguucuuggugcucuuggcu

SEQ ID NO: 25 - RNA, 23 nt, Artificial Sequence
uaguucuuggugcucuuggcuug

SEQ ID NO: 26 - RNA, 19 nt, Artificial Sequence
ccaagagcaccaagaacua

SEQ ID NO: 27 - RNA, 21 nt, Artificial Sequence
agccaagagcaccaagaacua

SEQ ID NO: 28 - RNA, 21 nt, Artificial Sequence
uaguucuuggugcucuuggcu

SEQ ID NO: 29 - RNA, 23 nt, Artificial Sequence
uaguucuuggugcucuuggcuug

SEQ ID NO: 30 - RNA, 21 nt, Artificial Sequence
uaguucuuggugcucuuggcu

SEQ ID NO: 31 - RNA, 23 nt, Artificial Sequence
uaguucuuggugcucuuggcuug

SEQ ID NO: 32 - RNA, 21 nt, Artificial Sequence
uaguucuuggugcucuuggcu

SEQ ID NO: 33 - RNA, 23 nt, Artificial Sequence
uaguucuuggugcucuuggcuug

SEQ ID NO: 34 - RNA, 21 nt, Artificial Sequence
uaguucuuggugcucuuggcu

SEQ ID NO: 35 - RNA, 23 nt, Artificial Sequence
uaguucuuggugcucuuggcuug

SEQ ID NO: 36 - RNA, 21 nt, Artificial Sequence
uaguucuuggugcucuuggcu

SEQ ID NO: 37 - RNA, 21 nt, Artificial Sequence
uaguucuuggugcucuuggcu

SEQ ID NO: 38 - RNA, 21 nt, Artificial Sequence
uaguucuuggugcucuuggcu

SEQ ID NO: 39 - RNA, 21 nt, Artificial Sequence
uaguucuuggugcucuuggcu

SEQ ID NO: 40 - RNA, 21 nt, Artificial Sequence
uaguucuuggugcucuuggcu

SEQ ID NO: 41 - RNA, 21 nt, Artificial Sequence
uaguucuuggugcucuuggcu

SEQ ID NO: 42 - RNA, 21 nt, Artificial Sequence
uaguucuuggugcucuuggcu

SEQ ID NO: 43 - RNA, 23 nt, Artificial Sequence
uaguucuuggugcucuuggcuug

SEQ ID NO: 44 - RNA, 23 nt, Artificial Sequence
uaguucuuggugcucuuggcuug

SEQ ID NO: 45 - RNA, 23 nt, Artificial Sequence
uaguucuuggugcucuuggcuug

SEQ ID NO: 46 - RNA, 21 nt, Artificial Sequence
uaguucuuggugcucuuggcu

SEQ ID NO: 47 - RNA, 21 nt, Artificial Sequence
agccaagagcaccaagaacua

SEQ ID NO: 48 - RNA, 23 nt, Artificial Sequence
uaguucuuggugcucuuggcuug

SEQ ID NO: 49 - RNA, 19 nt, Artificial Sequence
ccuugaggcauacuucaaa

SEQ ID NO: 50 - RNA, 21 nt, Artificial Sequence
uuugaaguaugccucaagguu

SEQ ID NO: 51 - RNA, 21 nt, Artificial Sequence
acauauuugaucagucuuuuu

SEQ ID NO: 52 - RNA, 23 nt, Artificial Sequence
aaaaagacugaucaaauauguug

SEQ ID NO: 53 - DNA, 18 bp, Artificial Sequence
accaactatacgctacat

SEQ ID NO: 54 - DNA, 18 bp, Artificial Sequence
cctcctgaataaccctct

SEQ ID NO: 55 - DNA, 19 bp, Artificial Sequence
ggtcggagtcaacggattt

SEQ ID NO: 56 - DNA, 19 bp, Artificial Sequence
ccagcatcgccccacttga

SEQ ID NO: 57 - DNA, 23 bp, Artificial Sequence
gaggagcagctaaccaacttaat

SEQ ID NO: 58 - DNA, 23 bp, Artificial Sequence
tctgcatgtgctgttgacttaat

SEQ ID NO: 59 - DNA, 24 bp, Artificial Sequence
aactttggcattgtggaagggctc

SEQ ID NO: 60 - DNA, 24 bp, Artificial Sequence
tggaagagtgggagttgctgttga

SEQ ID NO: 61 - DNA, 20 bp, Artificial Sequence
ctggtggtggcatgatgagt

SEQ ID NO: 62 - DNA, 21 bp, Artificial Sequence
ctcttctccgctctggcttag

SEQ ID NO: 63 - DNA, 20 bp, Artificial Sequence
gggagccaaaagggtcatca

SEQ ID NO: 64 - DNA, 20 bp, Artificial Sequence
cgtggactgtggtcatgagt